European Patent Specification EP 4 000 609 B1, published November 13, 2024. Title: Pharmaceutical compositions for preventing or treating bone diseases. Applicant: INDUSTRY FOUNDATION OF CHONNAM NATIONAL UNIVERSITY. The sequence listing filed with the application follows.

SEQUENCE LISTING (14 sequences)

SEQ ID NO: 1 - DNA, 20 bp, Artificial Sequence
  NFATc1 Forward primer
cccgtcacattctggtccat

SEQ ID NO: 2 - DNA, 23 bp, Artificial Sequence
  NFATc1 Reverse primer
caagtaaccgtgtagctccacaa

SEQ ID NO: 3 - DNA, 21 bp, Artificial Sequence
  CatK Forward primer
ggacgcagcgatgctaactaa

SEQ ID NO: 4 - DNA, 28 bp, Artificial Sequence
  CatK Reverse primer
cagagagaagggaagtagagttgtcact

SEQ ID NO: 5 - DNA, 21 bp, Artificial Sequence
  c-Fos Forward primer
cgaagggaacggaataagatg

SEQ ID NO: 6 - DNA, 20 bp, Artificial Sequence
  c- Fos Reverse primer
gctgccaaaataaactccag

SEQ ID NO: 7 - DNA, 20 bp, Artificial Sequence
  DC-STAMP Forward primer
gggagtcctgcaccatatgg

SEQ ID NO: 8 - DNA, 22 bp, Artificial Sequence
  DC-STAMP Reverse primer
aggccagtgctgactaggatga

SEQ ID NO: 9 - DNA, 23 bp, Artificial Sequence
  OC-STAMP Forward primer
cagagtgaccacctgaacaaaca

SEQ ID NO: 10 - DNA, 20 bp, Artificial Sequence
  OC-STAMP Reverse primer
tgcctgaggtccctgtgact

SEQ ID NO: 11 - DNA, 22 bp, Artificial Sequence
  TRAF6 Forward primer
aaagcgagagattctttccctg

SEQ ID NO: 12 - DNA, 22 bp, Artificial Sequence
  TRAF6 Reverse primer
actggggacaattcactagagc

SEQ ID NO: 13 - DNA, 19 bp, Artificial Sequence
  Acp5 Forward primer
cagctgtcctggctcaaaa

SEQ ID NO: 14 - DNA, 20 bp, Artificial Sequence
  Acp5 Reverse primer
acatagcccacaccgttctc